European Patent Application EP 4 403 214 A2, published July 24, 2024. Title: Methods of treating metabolic disorders with FGF21 variants. Applicant: Novartis AG. Application EP. The sequence listing filed with the application follows.

SEQUENCE LISTING (14 sequences)

SEQ ID NO: 1 - protein, 209 aa, Homo sapiens
MDSDETGFEHSGLWVSVLAGLLLGACQAHPIPDSSPLLQFGGQVRQRYLYTDDAQQTEAHLEIREDGTVGGAADQSPESLLQLKALKPGVIQILGVKTSRFLCQRPDGALYGSLHFDPEACSFRELLLEDGYNVYQSEAHGLPLHLPGNKSPHRDPAPRGPARFLPLPGLPPALPEPPGILAPQPPDVGSSDPLSMVGPSQGRSPSYAS

SEQ ID NO: 2 - DNA, 940 bp, Homo sapiens
  source 1..940: mol_type = genomic DNA
ctgtcagctgaggatccagccgaaagaggagccaggcactcaggccacctgagtctactcacctggacaactggaatctggcaccaattctaaaccactcagcttctccgagctcacaccccggagatcacctgaggacccgagccattgatggactcggacgagaccgggttcgagcactcaggactgtgggtttctgtgctggctggtcttctgctgggagcctgccaggcacaccccatccctgactccagtcctctcctgcaattcgggggccaagtccggcagcggtacctctacacagatgatgcccagcagacagaagcccacctggagatcagggaggatgggacggtggggggcgctgctgaccagagccccgaaagtctcctgcagctgaaagccttgaagccgggagttattcaaatcttgggagtcaagacatccaggttcctgtgccagcggccagatggggccctgtatggatcgctccactttgaccctgaggcctgcagcttccgggagctgcttcttgaggacggatacaatgtttaccagtccgaagcccacggcctcccgctgcacctgccagggaacaagtccccacaccgggaccctgcaccccgaggaccagctcgcttcctgccactaccaggcctgccccccgcactcccggagccacccggaatcctggccccccagccccccgatgtgggctcctcggaccctctgagcatggtgggaccttcccagggccgaagccccagctacgcttcctgaagccagaggctgtttactatgacatctcctctttatttattaggttatttatcttatttatttttttatttttcttacttgagataataaagagttccagaggagaaaaaaaaaaaaaaaaaaaaaaaaaaaaaaaaaaaaaaaaaaaaaaaaaaaaaaa

SEQ ID NO: 3 - protein, 181 aa, Homo sapiens
HPIPDSSPLLQFGGQVRQRYLYTDDAQQTEAHLEIREDGTVGGAADQSPESLLQLKALKPGVIQILGVKTSRFLCQRPDGALYGSLHFDPEACSFRELLLEDGYNVYQSEAHGLPLHLPGNKSPHRDPAPRGPARFLPLPGLPPALPEPPGILAPQPPDVGSSDPLSMVGPSQGRSPSYAS

SEQ ID NO: 4 - DNA, 546 bp, Homo sapiens
  source 1..546: mol_type = genomic DNA
caccccatccctgactccagtcctctcctgcaattcgggggccaagtccggcagcggtacctctacacagatgatgcccagcagacagaagcccacctggagatcagggaggatgggacggtggggggcgctgctgaccagagccccgaaagtctcctgcagctgaaagccttgaagccgggagttattcaaatcttgggagtcaagacatccaggttcctgtgccagcggccagatggggccctgtatggatcgctccactttgaccctgaggcctgcagcttccgggagctgcttcttgaggacggatacaatgtttaccagtccgaagcccacggcctcccgctgcacctgccagggaacaagtccccacaccgggaccctgcaccccgaggaccagctcgcttcctgccactaccaggcctgccccccgcactcccggagccacccggaatcctggccccccagccccccgatgtgggctcctcggaccctctgagcatggtgggaccttcccagggccgaagccccagctacgcttcctga

SEQ ID NO: 5-6 - skipped (2 entries)

SEQ ID NO: 7 - protein, 406 aa, synthetic construct
  REGION 1..406: note = Description of the artificial sequence: synthetic peptide
DKTHTCPPCPAPEAAGGPSVFLFPPKPKDTLMISRTPEVTCVVVDVSHEDPEVKFNWYVDGVEVHNAKTKPREEQYNSTYRVVSVLTVLHQDWLNGKEYKCKVSNKALPAPIEKTISKAKGQPREPQVYTLPPSREEMTKNQVSLTCLVKGFYPSDIAVEWESNGQPENNYKTTPPVLDSDGSFFLYSKLTVDKSRWQQGNVFSCSVMHEALHNHYTQKSLSLSPGKGSDSSPLLQFGGQVRQRYLYTDDAQQTEAHLEIREDGTVGGAADQSPESLLQLKALKPGVIQILGVKTSRFLCQRPDGALYGSLHFDPEACSFRELLLEDGYNVYQSEAHGLPLHLPGNKSPHRDPAPRGPARFLPLPGLPPALPEPPGILAPQPPDVGSSDPLSMVGPSQGRSPSYAS

SEQ ID NO: 8 - protein, 419 aa, synthetic construct
  REGION 1..419: note = Description of artificial sequence: synthetic peptide
DKTHTCPPCPAPEAAGGPSVFLFPPKPKDTLMISRTPEVTCVVVDVSHEDPEVKFNWYVDGVEVHNAKTKPREEQYNSTYRVVSVLTVLHQDWLNGKEYKCKVSNKALPAPIEKTISKAKGQPREPQVYTLPPSREEMTKNQVSLTCLVKGFYPSDIAVEWESNGQPENNYKTTPPVLDSDGSFFLYSKLTVDKSRWQQGNVFSCSVMHEALHNHYTQKSLSLSPGKGGGGSGGGGSGGGGSDSSPLLQFGGQVRQRYLYTDDAQQTEAHLEIREDGTVGGAADQSPESLLQLKALKPGVIQILGVKTSRFLCQRPDGALYGSLHFDPEACSFRELLLEDGYNVYQSEAHGLPLHLPGNKSPHRDPAPRGPARFLPLPGLPPALPEPPGILAPQPPDVGSSDPLSMVGPSQGRSPSYAS

SEQ ID NO: 9 - protein, 177 aa, synthetic construct
  REGION 1..177: note = Description of artificial sequence: synthetic peptide
DSSPLLQFGGQVRQRYLYTDDAQETEAHLEIREDGTVGGAAHQSPESLLELKALKPGVIQILGVKTSRFLCQKPDGALYGSLHFDPEACSFRELLLEDGYNVYQSEAHGLPLHLPGNRSPHCDPAPQGPARFLPLPGLPPALPEPPGILAPQPPDVGSSDPLAMVGPSQGRSPSYAS

SEQ ID NO: 10 - protein, 406 aa, synthetic construct
  REGION 1..406: note = Description of artificial sequence: synthetic peptide
DKTHTCPPCPAPEAAGGPSVFLFPPKPKDTLMISRTPEVTCVVVDVSHEDPEVKFNWYVDGVEVHNAKTKPREEQYNSTYRVVSVLTVLHQDWLNGKEYKCKVSNKALPAPIEKTISKAKGQPREPQVYTLPPSREEMTKNQVSLTCLVKGFYPSDIAVEWESNGQPENNYKTTPPVLDSDGSFFLYSKLTVDKSRWQQGNVFSCSVMHEALHNHYTQKSLSLSPGKGSDSSPLLQFGGQVRQRYLYTDDACQTEAHLEIREDGTVGGAADQSPESLLQLKALKPGVIQILGVKTSRFLCQRPDGTLYGSLHFDPEACSFRELLLEDGYNVYQSEAHGLPLHLPCNRSPHRDPASRGPARFLPLPGLPPALPEPPGILAPQPPDVGSSDPLAMVGGSQARSPSYAS

SEQ ID NO: 11 - protein, 406 aa, synthetic construct
  REGION 1..406: note = Description of artificial sequence: synthetic peptide
DKTHTCPPCPAPEAAGGPSVFLFPPKPKDTLMISRTPEVTCVVVDVSHEDPEVKFNWYVDGVEVHNAKTKPREEQYNSTYRVVSVLTVLHQDWLNGKEYKCKVSNKALPAPIEKTISKAKGQPREPQVYTLPPSREEMTKNQVSLTCLVKGFYPSDIAVEWESNGQPENNYKTTPPVLDSDGSFFLYSKLTVDKSRWQQGNVFSCSVMHEALHNHYTQKSLSLSPGKGSDSSPLLQFGGQVRQRYLYTDDACQTEAHLEIREDGTVGGAADQSPESLLQLKALKPGVIQILGVKTSRFLCQKPDGALYGSLHFDPEACSFRELLLEDGYNVYQSEAHGLPLHLPCNRSPHRDPASRGPARFLPLPGLPPALPEPPGILAPQPPDVGSSDPLAMVGGSQARSPSYAS

SEQ ID NO: 12 - protein, 419 aa, synthetic construct
  REGION 1..419: note = Description of artificial sequence: synthetic peptide
DKTHTCPPCPAPEAAGGPSVFLFPPKPKDTLMISRTPEVTCVVVDVSHEDPEVKFNWYVDGVEVHNAKTKPREEQYNSTYRVVSVLTVLHQDWLNGKEYKCKVSNKALPAPIEKTISKAKGQPREPQVYTLPPSREEMTKNQVSLTCLVKGFYPSDIAVEWESNGQPENNYKTTPPVLDSDGSFFLYSKLTVDKSRWQQGNVFSCSVMHEALHNHYTQKSLSLSPGKGGGGSGGGGSGGGGSDSSPLLQFGGQVRQRYLYTDDACQTEAHLEIREDGTVGGAADQSPESLLQLKALKPGVIQILGVKTSRFLCQKPDGALYGSLHFDPEACSFRELLLEDGYNVYQSEAHGLPLHLPCNRSPHRDPASRGPARFLPLPGLPPALPEPPGILAPQPPDVGSSDPLAMVGGSQARSPSYAS

SEQ ID NO: 13 - protein, 419 aa, synthetic construct
  REGION 1..419: note = Description of artificial sequence: synthetic peptide
DKTHTCPPCPAPEAAGGPSVFLFPPKPKDTLMISRTPEVTCVVVDVSHEDPEVKFNWYVDGVEVHNAKTKPREEQYNSTYRVVSVLTVLHQDWLNGKEYKCKVSNKALPAPIEKTISKAKGQPREPQVYTLPPSREEMTKNQVSLTCLVKGFYPSDIAVEWESNGQPENNYKTTPPVLDSDGSFFLYSKLTVDKSRWQQGNVFSCSVMHEALHNHYTQKSLSLSPGKGGGGSGGGGSGGGGSDSSPLLQFGGQVRQRYLYTDDACQTEAHLEIREDGTVGGAADQSPESLLQLKALKPGVIQILGVKTSRFLCQRPDGTLYGSLHFDPEACSFRELLLEDGYNVYQSEAHGLPLHLPCNRSPHRDPASRGPARFLPLPGLPPALPEPPGILAPQPPDVGSSDPLAMVGGSQARSPSYAS

SEQ ID NO: 14 - protein, 15 aa, synthetic construct
  REGION 1..15: note = Description of artificial sequence: synthetic peptide
GGGGSGGGGSGGGGS